European Patent Application EP 4 371 567 A1, published May 22, 2024. Title: AGENT FOR IMPROVING INTESTINAL FLORA. Applicant: AMANO ENZYME INC. HIROSHIMA UNIVERSITY. Application EP 22841878.6. The sequence listing filed with the application follows.

SEQUENCE LISTING (4 sequences)

SEQ ID NO: 1 - DNA, 17 bp, Artificial Sequence
  Forward primer for Bifidobacterium spp.
cgcgtcyggtgtgaaag

SEQ ID NO: 2 - DNA, 18 bp, Artificial Sequence
  Reverse primer for Bifidobacterium spp.
ccccacatccagcatcca

SEQ ID NO: 3 - DNA, 22 bp, Artificial Sequence
  Forward primer for Lactobacillus spp.
gaggcagcagtagggaatcttc

SEQ ID NO: 4 - DNA, 27 bp, Artificial Sequence
  Reverse primer for Lactobacillus spp.
ggccagttactacctctatccttcttc